European Patent Specification EP 3 690 038 B1, published July 29, 2026. Title: Antibody-Pyrrolobenzodiazepine Derivative Conjugate. Applicant: DAIICHI SANKYO COMPANY, LIMITED. The sequence listing filed with the application follows.

SEQUENCE LISTING (75 sequences)

SEQ ID NO: 1 - protein, 220 aa, Homo sapiens
  MISC_FEATURE: amino acid sequence of human CLDN6
MASAGMQILGVVLTLLGWVNGLVSCALPMWKVTAFIGNSIVVAQVVWEGLWMSCVVQSTGQMQCKVYDSLLALPQDLQAARALCVIALLVALFGLLVYLAGAKCTTCVEEKDSKARLVLTSGIVFVISGVLTLIPVCWTAHAIIRDFYNPLVAEAQKRELGASLYLGWAASGLLLLGGGLLCCTCPSGGSQGPSHYMARYSTSAPAISRGPSEYPTKNYV

SEQ ID NO: 2 - DNA, 663 bp, Homo sapiens
  misc_feature: nucleotide sequence of cDNA encoding amino acid sequence of human CLDN6
atggcctctgccggaatgcagatcctgggagtcgtcctgacactgctgggctgggtgaatggcctggtctcctgtgccctgcccatgtggaaggtgaccgctttcatcggcaacagcatcgtggtggcccaggtggtgtgggagggcctgtggatgtcctgcgtggtgcagagcaccggccagatgcagtgcaaggtgtacgactcactgctggcgctgccacaggacctgcaggctgcacgtgccctctgtgtcatcgccctccttgtggccctgttcggcttgctggtctaccttgctggggccaagtgtaccacctgtgtggaggagaaggattccaaggcccgcctggtgctcacctctgggattgtctttgtcatctcaggggtcctgacgctaatccccgtgtgctggacggcgcatgccatcatccgggacttctataaccccctggtggctgaggcccaaaagcgggagctgggggcctccctctacttgggctgggcggcctcaggccttttgttgctgggtggggggttgctgtgctgcacttgcccctcgggggggtcccagggccccagccattacatggcccgctactcaacatctgcccctgccatctctcgggggccctctgagtaccctaccaagaattacgtctga

SEQ ID NO: 3 - protein, 217 aa, Homo sapiens
  MISC_FEATURE: amino acid sequence of human CLDN9
MASTGLELLGMTLAVLGWLGTLVSCALPLWKVTAFIGNSIVVAQVVWEGLWMSCVVQSTGQMQCKVYDSLLALPQDLQAARALCVIALLLALLGLLVAITGAQCTTCVEDEGAKARIVLTAGVILLLAGILVLIPVCWTAHAIIQDFYNPLVAEALKRELGASLYLGWAAAALLMLGGGLLCCTCPPPQVERPRGPRLGYSIPSRSGASGLDKRDYV

SEQ ID NO: 4 - DNA, 654 bp, Homo sapiens
  misc_feature: nucleotide sequence of cDNA encoding amino acid sequence of human CLDN9
atggcttcgaccggcttagaactgctgggcatgaccctggctgtgctgggctggctggggaccctggtgtcctgcgccctgcccctgtggaaggtgaccgccttcatcggcaacagcatcgtggtggcccaggtggtgtgggagggcctgtggatgtcctgcgtggtgcagagcacgggccagatgcagtgcaaggtgtacgactcactgctggctctgccgcaggacctgcaggccgcacgtgccctctgtgtcattgccctcctgctggccctgcttggcctcctggtggccatcacaggtgcccagtgtaccacgtgtgtggaggacgaaggtgccaaggcccgtatcgtgctcaccgcgggggtcatcctcctcctcgccggcatcctggtgctcatccctgtgtgctggacggcgcacgccatcatccaggacttctacaaccccctggtggctgaggccctcaagcgggagctgggggcctccctctacctgggctgggcggcggctgcactgcttatgctgggcggggggctcctctgctgcacgtgccccccgccccaggtcgagcggccccgcggacctcggctgggctactccatcccctcccgctcgggtgcatctggactggacaagagggactacgtgtga

SEQ ID NO: 5 - protein, 11 aa, Mus musculus
  MISC_FEATURE: amino acid sequence of CDRL1 of B1 antibody light chain
RASQDINNYLN

SEQ ID NO: 6 - protein, 7 aa, Mus musculus
  MISC_FEATURE: amino acid sequence of CDRL2 of B1 antibody light chain
FTSRLHS

SEQ ID NO: 7 - protein, 9 aa, Mus musculus
  MISC_FEATURE: amino acid sequence of CDRL3 of B1 antibody light chain
QQGYPLPWT

SEQ ID NO: 8 - protein, 9 aa, Artificial Sequence
  humanized antibody
  MISC_FEATURE: amino acid sequence of CDRL3 of humanized B1 antibody light chain L4
QQGNTLPWT

SEQ ID NO: 9 - protein, 10 aa, Mus musculus
  MISC_FEATURE: amino acid sequence of CDRH1 of B1 antibody heavy chain
GYTFTEYTMH

SEQ ID NO: 10 - protein, 10 aa, Mus musculus
  MISC_FEATURE: amino acid sequence of CDRH2 of B1 antibody heavy chain
GVNPNSGDTS

SEQ ID NO: 11 - protein, 13 aa, Mus musculus
  MISC_FEATURE: amino acid sequence of CDRH3 of B1 antibody heavy chain
PGGYDVGYYAMDY

SEQ ID NO: 12 - protein, 11 aa, Mus musculus
  MISC_FEATURE: amino acid sequence of CDRL1 of C7 antibody light chain
RASQDINNYLN

SEQ ID NO: 13 - protein, 7 aa, Mus musculus
  MISC_FEATURE: amino acid sequence of CDRL2 of C7 antibody light chain
STSRLHS

SEQ ID NO: 14 - protein, 9 aa, Mus musculus
  MISC_FEATURE: amino acid sequence of CDRL3 of C7 antibody light chain
QQGYPLPWT

SEQ ID NO: 15 - protein, 10 aa, Mus musculus
  MISC_FEATURE: amino acid sequence of CDRH1 of C7 antibody heavy chain
GYTFTEYTMH

SEQ ID NO: 16 - protein, 10 aa, Mus musculus
  MISC_FEATURE: amino acid sequence of CDRH2 of C7 antibody heavy chain
GVNPNSGDTS

SEQ ID NO: 17 - protein, 13 aa, Mus musculus
  MISC_FEATURE: amino acid sequence of CDRH3 of C7 antibody heavy chain
PGGYDVGYYAMDY

SEQ ID NO: 18 - DNA, 321 bp, Mus musculus
  misc_feature: nucleotide sequence of cDNA encoding variable region of B1 antibody light chain
gatatccagatgacacagactgcatcctccctgtctgcctctcttggagacagagtcaccatcagttgcagggcaagtcaggacattaacaattatttaaactggtatcagcagaaaccagatggaactgttaaactcctgatctacttcacatcaagattacactcaggagtcccatcaaggttcagtggcagtgggtctggaacacattattctctcaccattactaacctggaacaagaagatattgccacttacttttgccaacagggttatccgcttccgtggacgttcggtggaggcaccaaactggaaatcaaa

SEQ ID NO: 19 - protein, 107 aa, Mus musculus
  MISC_FEATURE: amino acid sequence of variable region of B1 antibody light chain
DIQMTQTASSLSASLGDRVTISCRASQDINNYLNWYQQKPDGTVKLLIYFTSRLHSGVPSRFSGSGSGTHYSLTITNLEQEDIATYFCQQGYPLPWTFGGGTKLEIK

SEQ ID NO: 20 - DNA, 366 bp, Mus musculus
  misc_feature: nucleotide sequence of cDNA encoding variable region of B1 antibody heavy chain
gaggtccagcttcaacagtctggacctgaactggtgaagcctggggcttcagtgaagatatcctgcaagacttctggatacacattcactgaatacaccatgcactgggtgcagcagagccatggaaagagccttgagtggattggaggtgttaatcctaatagtggtgatactagctacaaccagaagttcaagggcaaggccacattgactgttgacaagtcctccagcacagcctacatggagctccgcagcctgacatctgaggattctgcagtctattactgtgcaagacccggggggtacgacgtgggttactatgctatggactactggggtcaaggaacctcagtcaccgtctcctca

SEQ ID NO: 21 - protein, 122 aa, Mus musculus
  MISC_FEATURE: amino acid sequence of variable region of B1 antibody heavy chain
EVQLQQSGPELVKPGASVKISCKTSGYTFTEYTMHWVQQSHGKSLEWIGGVNPNSGDTSYNQKFKGKATLTVDKSSSTAYMELRSLTSEDSAVYYCARPGGYDVGYYAMDYWGQGTSVTVSS

SEQ ID NO: 22 - DNA, 321 bp, Mus musculus
  misc_feature: nucleotide sequence of cDNA encoding variable region of C7 antibody light chain
gatatccagatgacacagactgcatcctccctgtctgcctctcttggagacagagtcaccatcagttgcagggcaagtcaggacattaacaattatttaaactggtatcagcagaaaccagatggaactgttaaactcctgatctactccacatcaagattacactcaggagtcccatcaaggttcagtggcagtgggtctggaacacattattctctcaccattactcacctggaacaagaagatattgccacttacttttgccaacagggttatccgcttccgtggacgttcggtggaggcaccaaactggaaatcaaa

SEQ ID NO: 23 - protein, 107 aa, Mus musculus
  MISC_FEATURE: amino acid sequence of variable region of C7 antibody light chain
DIQMTQTASSLSASLGDRVTISCRASQDINNYLNWYQQKPDGTVKLLIYSTSRLHSGVPSRFSGSGSGTHYSLTITHLEQEDIATYFCQQGYPLPWTFGGGTKLEIK

SEQ ID NO: 24 - DNA, 366 bp, Mus musculus; identical to SEQ ID NO: 20
  misc_feature: nucleotide sequence of cDNA encoding variable region of C7 antibody heavy chain

SEQ ID NO: 25 - protein, 122 aa, Mus musculus; identical to SEQ ID NO: 21
  MISC_FEATURE: amino acid sequence of variable region of C7 antibody heavy chain

SEQ ID NO: 26 - DNA, 449 bp, Homo sapiens
  misc_feature: DNA fragment comprising DNA sequence encoding human light chain signal sequence and human  È chain constant region
gcctccggactctagagccaccatggtgctgcagacccaggtgttcatctccctgctgctgtggatctccggcgcgtacggcgatatcgtgatgattaaacgtacggtggccgccccctccgtgttcatcttccccccctccgacgagcagctgaagtccggcaccgcctccgtggtgtgcctgctgaataacttctaccccagagaggccaaggtgcagtggaaggtggacaacgccctgcagtccgggaactcccaggagagcgtgaccgagcaggacagcaaggacagcacctacagcctgagcagcaccctgaccctgagcaaagccgactacgagaagcacaaggtgtacgcctgcgaggtgacccaccagggcctgagctcccccgtcaccaagagcttcaacaggggggagtgttaggggcccgtttaaacgggggaggcta

SEQ ID NO: 27 - DNA, 1137 bp, Homo sapiens
  misc_feature: DNA fragment comprising DNA sequence encoding human heavy chain signal sequence and human IgG1 LALA constant region
ccagcctccggactctagagccaccatgaaacacctgtggttcttcctcctgctggtggcagctcccagatgggtgctgagccaggtgcaattgtgcaggcggttagctcagcctccaccaagggcccaagcgtcttccccctggcaccctcctccaagagcacctctggcggcacagccgccctgggctgcctggtcaaggactacttccccgaacccgtgaccgtgagctggaactcaggcgccctgaccagcggcgtgcacaccttccccgctgtcctgcagtcctcaggactctactccctcagcagcgtggtgaccgtgccctccagcagcttgggcacccagacctacatctgcaacgtgaatcacaagcccagcaacaccaaggtggacaagagagttgagcccaaatcttgtgacaaaactcacacatgcccaccctgcccagcacctgaagccgcggggggaccctcagtcttcctcttccccccaaaacccaaggacaccctcatgatctcccggacccctgaggtcacatgcgtggtggtggacgtgagccacgaagaccctgaggtcaagttcaactggtacgtggacggcgtggaggtgcataatgccaagacaaagccccgggaggagcagtacaacagcacgtaccgggtggtcagcgtcctcaccgtcctgcaccaggactggctgaatggcaaggagtacaagtgcaaggtctccaacaaagccctcccagcccccatcgagaaaaccatctccaaagccaaaggccagccccgggaaccacaggtgtacaccctgcccccatcccgggaggagatgaccaagaaccaggtcagcctgacctgcctggtcaaaggcttctatcccagcgacatcgccgtggagtgggagagcaatggccagcccgagaacaactacaagaccacccctcccgtgctggactccgacggctccttcttcctctacagcaagctcaccgtggacaagagcaggtggcagcagggcaacgtcttctcatgctccgtgatgcatgaggctctgcacaaccactacacccagaagagcctctccctgtctcccggcaaatgagatatcgggcccgtttaaacgggggaggctaac

SEQ ID NO: 28 - protein, 234 aa, Artificial Sequence
  chimeric antibody
  MISC_FEATURE: amino acid sequence of chB1 light chain
MVLQTQVFISLLLWISGAYGDIQMTQTASSLSASLGDRVTISCRASQDINNYLNWYQQKPDGTVKLLIYFTSRLHSGVPSRFSGSGSGTHYSLTITNLEQEDIATYFCQQGYPLPWTFGGGTKLEIKRAVAAPSVFIFPPSDEQLKSGTASVVCLLNNFYPREAKVQWKVDNALQSGNSQESVTEQDSKDSTYSLSSTLTLSKADYEKHKVYACEVTHQGLSSPVTKSFNRGEC

SEQ ID NO: 29 - DNA, 752 bp, Artificial Sequence
  chimeric antibody
  misc_feature: DNA fragment comprising DNA sequence encoding amino acid sequence of chB1 light chain
ccagcctccggactctagagccaccatggtgctgcagacccaggtgttcatcagcctgctgctgtggatcagcggcgcctacggcgacatccagatgacccagacagccagcagcctgagcgccagcctgggcgatagagtgaccatcagctgcagagccagccaggacatcaacaactacctgaactggtatcagcagaaacccgacggcaccgtgaagctgctgatctacttcaccagcagactgcacagcggcgtgcccagcagattttctggcagcggctctggcacccactacagcctgaccatcaccaacctggaacaggaagatatcgctacctacttctgtcagcaaggctaccccctgccctggacctttggcggcggaacaaagctggaaatcaagcgggccgtggccgctccctccgtgttcatctttccacccagcgacgagcagctgaagtccggcacagctagcgtcgtgtgcctgctgaacaacttctacccccgcgaggccaaggtgcagtggaaggtggacaatgccctgcagagcggcaacagccaggaaagcgtgaccgagcaggacagcaaggactccacctactccctgagcagcaccctgaccctgagcaaggccgactacgagaagcacaaggtgtacgcctgcgaagtgacccaccagggcctgtctagccccgtgaccaagagcttcaaccggggcgagtgttgagtttaaacgggggaggctaact

SEQ ID NO: 30 - protein, 107 aa, Artificial Sequence; identical to SEQ ID NO: 19
  chimeric antibody
  MISC_FEATURE: amino acid sequence of variable region of chB1 light chain

SEQ ID NO: 31 - DNA, 321 bp, Artificial Sequence
  chimeric antibody
  misc_feature: nucleotide sequence encoding amino acid sequence of variable region of chB1 light chain
gacatccagatgacccagacagccagcagcctgagcgccagcctgggcgatagagtgaccatcagctgcagagccagccaggacatcaacaactacctgaactggtatcagcagaaacccgacggcaccgtgaagctgctgatctacttcaccagcagactgcacagcggcgtgcccagcagattttctggcagcggctctggcacccactacagcctgaccatcaccaacctggaacaggaagatatcgctacctacttctgtcagcaaggctaccccctgccctggacctttggcggcggaacaaagctggaaatcaag

SEQ ID NO: 32 - protein, 471 aa, Artificial Sequence
  chimeric antibody
  MISC_FEATURE: amino acid sequence of chB1 heavy chain
MKHLWFFLLLVAAPRWVLSEVQLQQSGPELVKPGASVKISCKTSGYTFTEYTMHWVQQSHGKSLEWIGGVNPNSGDTSYNQKFKGKATLTVDKSSSTAYMELRSLTSEDSAVYYCARPGGYDVGYYAMDYWGQGTSVTVSSASTKGPSVFPLAPSSKSTSGGTAALGCLVKDYFPEPVTVSWNSGALTSGVHTFPAVLQSSGLYSLSSVVTVPSSSLGTQTYICNVNHKPSNTKVDKRVEPKSCDKTHTCPPCPAPEAAGGPSVFLFPPKPKDTLMISRTPEVTCVVVDVSHEDPEVKFNWYVDGVEVHNAKTKPREEQYNSTYRVVSVLTVLHQDWLNGKEYKCKVSNKALPAPIEKTISKAKGQPREPQVYTLPPSREEMTKNQVSLTCLVKGFYPSDIAVEWESNGQPENNYKTTPPVLDSDGSFFLYSKLTVDKSRWQQGNVFSCSVMHEALHNHYTQKSLSLSPGK

SEQ ID NO: 33 - DNA, 1413 bp, Artificial Sequence
  chimeric antibody
  misc_feature: nucleotide sequence encoding chB1 heavy chain
atgaaacacctgtggttcttcctcctgctggtggcagctcccagatgggtgctgagcgaagtgcagctgcagcagtctggccccgagctcgtgaaacctggcgcctccgtgaagatcagctgcaagaccagcggctacaccttcaccgagtacaccatgcactgggtgcagcagagccacggcaagagcctggaatggatcggcggcgtgaaccccaacagcggcgacaccagctacaaccagaagttcaagggcaaggccaccctgaccgtggacaagagcagcagcaccgcctacatggaactgcggagcctgaccagcgaggacagcgccgtgtactactgtgccagacctggcggctacgacgtgggctactacgccatggattactggggccagggcaccagcgtgaccgtcagctcagcctccaccaagggcccaagcgtcttccccctggcaccctcctccaagagcacctctggcggcacagccgccctgggctgcctggtcaaggactacttccccgaacccgtgaccgtgagctggaactcaggcgccctgaccagcggcgtgcacaccttccccgctgtcctgcagtcctcaggactctactccctcagcagcgtggtgaccgtgccctccagcagcttgggcacccagacctacatctgcaacgtgaatcacaagcccagcaacaccaaggtggacaagagagttgagcccaaatcttgtgacaaaactcacacatgcccaccctgcccagcacctgaagccgcggggggaccctcagtcttcctcttccccccaaaacccaaggacaccctcatgatctcccggacccctgaggtcacatgcgtggtggtggacgtgagccacgaagaccctgaggtcaagttcaactggtacgtggacggcgtggaggtgcataatgccaagacaaagccccgggaggagcagtacaacagcacgtaccgggtggtcagcgtcctcaccgtcctgcaccaggactggctgaatggcaaggagtacaagtgcaaggtctccaacaaagccctcccagcccccatcgagaaaaccatctccaaagccaaaggccagccccgggaaccacaggtgtacaccctgcccccatcccgggaggagatgaccaagaaccaggtcagcctgacctgcctggtcaaaggcttctatcccagcgacatcgccgtggagtgggagagcaatggccagcccgagaacaactacaagaccacccctcccgtgctggactccgacggctccttcttcctctacagcaagctcaccgtggacaagagcaggtggcagcagggcaacgtcttctcatgctccgtgatgcatgaggctctgcacaaccactacacccagaagagcctctccctgtctcccggcaaa

SEQ ID NO: 34 - protein, 122 aa, Artificial Sequence; identical to SEQ ID NO: 21
  chimeric antibody
  MISC_FEATURE: amino acid sequence of variable region of chB1 heavy chain

SEQ ID NO: 35 - DNA, 366 bp, Artificial Sequence
  chimeric antibody
  misc_feature: nucleotide sequence encoding variable region of chB1 heavy chain
gaagtgcagctgcagcagtctggccccgagctcgtgaaacctggcgcctccgtgaagatcagctgcaagaccagcggctacaccttcaccgagtacaccatgcactgggtgcagcagagccacggcaagagcctggaatggatcggcggcgtgaaccccaacagcggcgacaccagctacaaccagaagttcaagggcaaggccaccctgaccgtggacaagagcagcagcaccgcctacatggaactgcggagcctgaccagcgaggacagcgccgtgtactactgtgccagacctggcggctacgacgtgggctactacgccatggattactggggccagggcaccagcgtgaccgtcagctca

SEQ ID NO: 36 - protein, 234 aa, Artificial Sequence
  humanized antibody
  MISC_FEATURE: amino acid sequence of humanized antibody light chain hL1
MVLQTQVFISLLLWISGAYGDIQMTQSPSSLSASVGDRVTITCRASQDINNYLNWYQQKPGKAPKLLIYFTSRLHSGVPSRFSGSGSGTDYTLTISSLQPEDFATYYCQQGYPLPWTFGQGTKVEIKRTVAAPSVFIFPPSDEQLKSGTASVVCLLNNFYPREAKVQWKVDNALQSGNSQESVTEQDSKDSTYSLSSTLTLSKADYEKHKVYACEVTHQGLSSPVTKSFNRGEC

SEQ ID NO: 37 - DNA, 702 bp, Artificial Sequence
  humanized antibody
  misc_feature: nucleotide sequence encoding humanized antibody light chain hL1
atggtgctgcagacccaggtgttcatctccctgctgctgtggatctccggcgcgtacggcgacatccagatgacccagagccctagcagcctgagcgccagcgtgggcgacagagtgaccatcacctgtagagccagccaggacatcaacaactacctgaactggtatcagcagaagcccggcaaggcccccaagctgctgatctacttcaccagcagactgcacagcggcgtgcccagcagattttctggcagcggctccggcaccgactacaccctgacaatcagcagcctgcagcccgaggacttcgccacctactactgccagcagggctaccccctgccttggacatttggccagggcaccaaggtggaaatcaagcgtacggtggccgccccctccgtgttcatcttccccccctccgacgagcagctgaagtccggcaccgcctccgtggtgtgcctgctgaataacttctaccccagagaggccaaggtgcagtggaaggtggacaacgccctgcagtccgggaactcccaggagagcgtgaccgagcaggacagcaaggacagcacctacagcctgagcagcaccctgaccctgagcaaagccgactacgagaagcacaaggtgtacgcctgcgaggtgacccaccagggcctgagctcccccgtcaccaagagcttcaacaggggggagtgt

SEQ ID NO: 38 - protein, 107 aa, Artificial Sequence
  humanized antibody
  MISC_FEATURE: amino acid sequence of variable region of humanized antibody light chain hL1
DIQMTQSPSSLSASVGDRVTITCRASQDINNYLNWYQQKPGKAPKLLIYFTSRLHSGVPSRFSGSGSGTDYTLTISSLQPEDFATYYCQQGYPLPWTFGQGTKVEIK

SEQ ID NO: 39 - DNA, 321 bp, Artificial Sequence
  humanized antibody
  misc_feature: nucleotide sequence encoding variable region of humanized antibody light chain hL1
gacatccagatgacccagagccctagcagcctgagcgccagcgtgggcgacagagtgaccatcacctgtagagccagccaggacatcaacaactacctgaactggtatcagcagaagcccggcaaggcccccaagctgctgatctacttcaccagcagactgcacagcggcgtgcccagcagattttctggcagcggctccggcaccgactacaccctgacaatcagcagcctgcagcccgaggacttcgccacctactactgccagcagggctaccccctgccttggacatttggccagggcaccaaggtggaaatcaag

SEQ ID NO: 40 - protein, 234 aa, Artificial Sequence
  humanized antibody
  MISC_FEATURE: amino acid sequence of humanized antibody light chain hL2
MVLQTQVFISLLLWISGAYGDIQMTQSPSSLSASVGDRVTITCRASQDINNYLNWYQQKPGKAVKLLIYFTSRLHSGVPSRFSGSGSGTHYTLTISSLQPEDFATYYCQQGYPLPWTFGQGTKVEIKRTVAAPSVFIFPPSDEQLKSGTASVVCLLNNFYPREAKVQWKVDNALQSGNSQESVTEQDSKDSTYSLSSTLTLSKADYEKHKVYACEVTHQGLSSPVTKSFNRGEC

SEQ ID NO: 41 - DNA, 702 bp, Artificial Sequence
  humanized antibody
  misc_feature: nucleotide sequence encoding humanized antibody light chain hL2
atggtgctgcagacccaggtgttcatctccctgctgctgtggatctccggcgcgtacggcgacatccagatgacccagagccctagcagcctgagcgccagcgtgggcgacagagtgaccatcacctgtagagccagccaggacatcaacaactacctgaactggtatcagcagaaacccggcaaggccgtgaagctgctgatctacttcaccagcagactgcacagcggcgtgcccagcagattttctggcagcggctctggcacccactacaccctgacaatcagcagcctgcagcccgaggacttcgccacctactactgccagcagggctaccccctgccttggacatttggccagggcaccaaggtggaaatcaagcgtacggtggccgccccctccgtgttcatcttccccccctccgacgagcagctgaagtccggcaccgcctccgtggtgtgcctgctgaataacttctaccccagagaggccaaggtgcagtggaaggtggacaacgccctgcagtccgggaactcccaggagagcgtgaccgagcaggacagcaaggacagcacctacagcctgagcagcaccctgaccctgagcaaagccgactacgagaagcacaaggtgtacgcctgcgaggtgacccaccagggcctgagctcccccgtcaccaagagcttcaacaggggggagtgt

SEQ ID NO: 42 - protein, 107 aa, Artificial Sequence
  humanized antibody
  MISC_FEATURE: amino acid sequence of variable region of humanized antibody light chain hL2
DIQMTQSPSSLSASVGDRVTITCRASQDINNYLNWYQQKPGKAVKLLIYFTSRLHSGVPSRFSGSGSGTHYTLTISSLQPEDFATYYCQQGYPLPWTFGQGTKVEIK

SEQ ID NO: 43 - DNA, 321 bp, Artificial Sequence
  humanized antibody
  misc_feature: nucleotide sequence encoding variable region of humanized antibody light chain hL2
gacatccagatgacccagagccctagcagcctgagcgccagcgtgggcgacagagtgaccatcacctgtagagccagccaggacatcaacaactacctgaactggtatcagcagaaacccggcaaggccgtgaagctgctgatctacttcaccagcagactgcacagcggcgtgcccagcagattttctggcagcggctctggcacccactacaccctgacaatcagcagcctgcagcccgaggacttcgccacctactactgccagcagggctaccccctgccttggacatttggccagggcaccaaggtggaaatcaag

SEQ ID NO: 44 - protein, 234 aa, Artificial Sequence
  humanized antibody
  MISC_FEATURE: amino acid sequence of humanized antibody light chain hL3
MVLQTQVFISLLLWISGAYGDIQMTQSPSSLSASVGDRVTITCRASQDINNYLNWYQQKPGGAVKLLIYFTSRLHSGVPSRFSGSGSGTDYTLTISSLQPEDFATYYCQQGYPLPWTFGGGTKVEIKRTVAAPSVFIFPPSDEQLKSGTASVVCLLNNFYPREAKVQWKVDNALQSGNSQESVTEQDSKDSTYSLSSTLTLSKADYEKHKVYACEVTHQGLSSPVTKSFNRGEC

SEQ ID NO: 45 - DNA, 702 bp, Artificial Sequence
  humanized antibody
  misc_feature: nucleotide sequence encoding humanized antibody light chain hL3
atggtgctgcagacccaggtgttcatctccctgctgctgtggatctccggcgcgtacggcgacatccagatgacccagagccctagcagcctgagcgccagcgtgggcgacagagtgaccatcacctgtagagccagccaggacatcaacaactacctgaactggtatcagcagaaacccggcggagccgtgaagctgctgatctacttcaccagcagactgcacagcggcgtgcccagcagattttctggcagcggctccggcaccgactacaccctgacaatcagcagcctgcagcccgaggacttcgccacctactactgccagcagggctaccccctgccctggacatttggcggcggaacaaaggtggaaatcaagcgtacggtggccgccccctccgtgttcatcttccccccctccgacgagcagctgaagtccggcaccgcctccgtggtgtgcctgctgaataacttctaccccagagaggccaaggtgcagtggaaggtggacaacgccctgcagtccgggaactcccaggagagcgtgaccgagcaggacagcaaggacagcacctacagcctgagcagcaccctgaccctgagcaaagccgactacgagaagcacaaggtgtacgcctgcgaggtgacccaccagggcctgagctcccccgtcaccaagagcttcaacaggggggagtgt

SEQ ID NO: 46 - protein, 107 aa, Artificial Sequence
  humanized antibody
  MISC_FEATURE: amino acid sequence of variable region of humanized antibody light chain hL3
DIQMTQSPSSLSASVGDRVTITCRASQDINNYLNWYQQKPGGAVKLLIYFTSRLHSGVPSRFSGSGSGTDYTLTISSLQPEDFATYYCQQGYPLPWTFGGGTKVEIK

SEQ ID NO: 47 - DNA, 321 bp, Artificial Sequence
  humanized antibody
  misc_feature: nucleotide sequence encoding variable region of humanized antibody light chain hL3
gacatccagatgacccagagccctagcagcctgagcgccagcgtgggcgacagagtgaccatcacctgtagagccagccaggacatcaacaactacctgaactggtatcagcagaaacccggcggagccgtgaagctgctgatctacttcaccagcagactgcacagcggcgtgcccagcagattttctggcagcggctccggcaccgactacaccctgacaatcagcagcctgcagcccgaggacttcgccacctactactgccagcagggctaccccctgccctggacatttggcggcggaacaaaggtggaaatcaag

SEQ ID NO: 48 - protein, 234 aa, Artificial Sequence
  humanized antibody
  MISC_FEATURE: amino acid sequence of humanized antibody light chain hL4
MVLQTQVFISLLLWISGAYGDIQMTQSPSSLSASVGDRVTITCRASQDINNYLNWYQQKPGGAVKLLIYFTSRLHSGVPSRFSGSGSGTDYTLTISSLQPEDFATYYCQQGNTLPWTFGGGTKVEIKRTVAAPSVFIFPPSDEQLKSGTASVVCLLNNFYPREAKVQWKVDNALQSGNSQESVTEQDSKDSTYSLSSTLTLSKADYEKHKVYACEVTHQGLSSPVTKSFNRGEC

SEQ ID NO: 49 - DNA, 702 bp, Artificial Sequence
  humanized antibody
  misc_feature: nucleotide sequence encoding humanized antibody light chain hL4
atggtgctgcagacccaggtgttcatctccctgctgctgtggatctccggcgcgtacggcgacatccagatgacccagagccctagcagcctgagcgccagcgtgggcgacagagtgaccatcacctgtagagccagccaggacatcaacaactacctgaactggtatcagcagaaacccggcggagccgtgaagctgctgatctacttcaccagcagactgcacagcggcgtgcccagcagattttctggcagcggctccggcaccgactacaccctgacaatcagcagcctgcagcccgaggacttcgccacctactactgccagcagggcaacaccctgccctggacatttggcggaggcaccaaggtggaaatcaagcgtacggtggccgccccctccgtgttcatcttccccccctccgacgagcagctgaagtccggcaccgcctccgtggtgtgcctgctgaataacttctaccccagagaggccaaggtgcagtggaaggtggacaacgccctgcagtccgggaactcccaggagagcgtgaccgagcaggacagcaaggacagcacctacagcctgagcagcaccctgaccctgagcaaagccgactacgagaagcacaaggtgtacgcctgcgaggtgacccaccagggcctgagctcccccgtcaccaagagcttcaacaggggggagtgt

SEQ ID NO: 50 - protein, 107 aa, Artificial Sequence
  humanized antibody
  MISC_FEATURE: amino acid sequence of variable region of humanized antibody light chain hL4
DIQMTQSPSSLSASVGDRVTITCRASQDINNYLNWYQQKPGGAVKLLIYFTSRLHSGVPSRFSGSGSGTDYTLTISSLQPEDFATYYCQQGNTLPWTFGGGTKVEIK

SEQ ID NO: 51 - DNA, 321 bp, Artificial Sequence
  humanized antibody
  misc_feature: nucleotide sequence encoding variable region of humanized antibody light chain hL4
gacatccagatgacccagagccctagcagcctgagcgccagcgtgggcgacagagtgaccatcacctgtagagccagccaggacatcaacaactacctgaactggtatcagcagaaacccggcggagccgtgaagctgctgatctacttcaccagcagactgcacagcggcgtgcccagcagattttctggcagcggctccggcaccgactacaccctgacaatcagcagcctgcagcccgaggacttcgccacctactactgccagcagggcaacaccctgccctggacatttggcggaggcaccaaggtggaaatcaag

SEQ ID NO: 52 - protein, 471 aa, Artificial Sequence
  humanized antibody
  MISC_FEATURE: amino acid sequence of humanized antibody heavy chain hH1
MKHLWFFLLLVAAPRWVLSQVQLVQSGAEVKKPGASVKVSCKASGYTFTEYTMHWVRQAPGQGLEWMGGVNPNSGDTSYAQKFQGRVTITADTSTSTAYMELSSLRSEDTAVYYCARPGGYDVGYYAMDYWGQGTLVTVSSASTKGPSVFPLAPSSKSTSGGTAALGCLVKDYFPEPVTVSWNSGALTSGVHTFPAVLQSSGLYSLSSVVTVPSSSLGTQTYICNVNHKPSNTKVDKRVEPKSCDKTHTCPPCPAPEAAGGPSVFLFPPKPKDTLMISRTPEVTCVVVDVSHEDPEVKFNWYVDGVEVHNAKTKPREEQYNSTYRVVSVLTVLHQDWLNGKEYKCKVSNKALPAPIEKTISKAKGQPREPQVYTLPPSREEMTKNQVSLTCLVKGFYPSDIAVEWESNGQPENNYKTTPPVLDSDGSFFLYSKLTVDKSRWQQGNVFSCSVMHEALHNHYTQKSLSLSPGK

SEQ ID NO: 53 - DNA, 1413 bp, Artificial Sequence
  humanized antibody
  misc_feature: nucleotide sequence encoding humanized antibody heavy chain hH1
atgaaacacctgtggttcttcctcctgctggtggcagctcccagatgggtgctgagccaggtgcagctggtgcagtctggcgccgaagtgaagaaaccaggcgccagcgtgaaggtgtcctgcaaggccagcggctacacctttaccgagtacaccatgcactgggtgcgccaggctccaggccagggactggaatggatgggcggcgtgaaccccaacagcggcgatacaagctacgcccagaaattccagggcagagtgaccatcaccgccgacaccagcacctccaccgcctacatggaactgagcagcctgcggagcgaggacaccgccgtgtactactgtgctagacctggcggctacgacgtgggctactacgccatggattactggggccagggcaccctcgtgaccgtcagctcagcctccaccaagggcccaagcgtcttccccctggcaccctcctccaagagcacctctggcggcacagccgccctgggctgcctggtcaaggactacttccccgaacccgtgaccgtgagctggaactcaggcgccctgaccagcggcgtgcacaccttccccgctgtcctgcagtcctcaggactctactccctcagcagcgtggtgaccgtgccctccagcagcttgggcacccagacctacatctgcaacgtgaatcacaagcccagcaacaccaaggtggacaagagagttgagcccaaatcttgtgacaaaactcacacatgcccaccctgcccagcacctgaagccgcggggggaccctcagtcttcctcttccccccaaaacccaaggacaccctcatgatctcccggacccctgaggtcacatgcgtggtggtggacgtgagccacgaagaccctgaggtcaagttcaactggtacgtggacggcgtggaggtgcataatgccaagacaaagccccgggaggagcagtacaacagcacgtaccgggtggtcagcgtcctcaccgtcctgcaccaggactggctgaatggcaaggagtacaagtgcaaggtctccaacaaagccctcccagcccccatcgagaaaaccatctccaaagccaaaggccagccccgggaaccacaggtgtacaccctgcccccatcccgggaggagatgaccaagaaccaggtcagcctgacctgcctggtcaaaggcttctatcccagcgacatcgccgtggagtgggagagcaatggccagcccgagaacaactacaagaccacccctcccgtgctggactccgacggctccttcttcctctacagcaagctcaccgtggacaagagcaggtggcagcagggcaacgtcttctcatgctccgtgatgcatgaggctctgcacaaccactacacccagaagagcctctccctgtctcccggcaaa

SEQ ID NO: 54 - protein, 122 aa, Artificial Sequence
  humanized antibody
  MISC_FEATURE: amino acid sequence of variable region of humanized antibody heavy chain hH1
QVQLVQSGAEVKKPGASVKVSCKASGYTFTEYTMHWVRQAPGQGLEWMGGVNPNSGDTSYAQKFQGRVTITADTSTSTAYMELSSLRSEDTAVYYCARPGGYDVGYYAMDYWGQGTLVTVSS

SEQ ID NO: 55 - DNA, 366 bp, Artificial Sequence
  humanized antibody
  misc_feature: nucleotide sequence encoding variable region of humanized antibody heavy chain hH1
caggtgcagctggtgcagtctggcgccgaagtgaagaaaccaggcgccagcgtgaaggtgtcctgcaaggccagcggctacacctttaccgagtacaccatgcactgggtgcgccaggctccaggccagggactggaatggatgggcggcgtgaaccccaacagcggcgatacaagctacgcccagaaattccagggcagagtgaccatcaccgccgacaccagcacctccaccgcctacatggaactgagcagcctgcggagcgaggacaccgccgtgtactactgtgctagacctggcggctacgacgtgggctactacgccatggattactggggccagggcaccctcgtgaccgtcagctca

SEQ ID NO: 56 - protein, 471 aa, Artificial Sequence
  humanized antibody
  MISC_FEATURE: amino acid sequence of humanized antibody heavy chain hH2
MKHLWFFLLLVAAPRWVLSEVQLVQSGAEVKKPGASVKVSCKTSGYTFTEYTMHWVRQAPGKSLEWMGGVNPNSGDTSYAQKFQGRVTITADTSTSTAYMELSSLRSEDTAVYYCARPGGYDVGYYAMDYWGQGTLVTVSSASTKGPSVFPLAPSSKSTSGGTAALGCLVKDYFPEPVTVSWNSGALTSGVHTFPAVLQSSGLYSLSSVVTVPSSSLGTQTYICNVNHKPSNTKVDKRVEPKSCDKTHTCPPCPAPEAAGGPSVFLFPPKPKDTLMISRTPEVTCVVVDVSHEDPEVKFNWYVDGVEVHNAKTKPREEQYNSTYRVVSVLTVLHQDWLNGKEYKCKVSNKALPAPIEKTISKAKGQPREPQVYTLPPSREEMTKNQVSLTCLVKGFYPSDIAVEWESNGQPENNYKTTPPVLDSDGSFFLYSKLTVDKSRWQQGNVFSCSVMHEALHNHYTQKSLSLSPGK

SEQ ID NO: 57 - DNA, 1413 bp, Artificial Sequence
  humanized antibody
  misc_feature: nucleotide sequence encoding humanized antibody heavy chain hH2
atgaaacacctgtggttcttcctcctgctggtggcagctcccagatgggtgctgagcgaagtgcagctggtgcagtctggcgccgaagtgaagaaaccaggcgccagcgtgaaggtgtcctgcaagaccagcggctacacctttaccgagtacaccatgcactgggtgcgccaggcccctggcaagagcctggaatggatgggcggcgtgaaccccaacagcggcgatacaagctacgcccagaaattccagggcagagtgaccatcaccgccgacaccagcacctccaccgcctacatggaactgagcagcctgcggagcgaggacaccgccgtgtactactgtgctagacctggcggctacgacgtgggctactacgccatggattactggggccagggcaccctcgtgaccgtcagctcagcctccaccaagggcccaagcgtcttccccctggcaccctcctccaagagcacctctggcggcacagccgccctgggctgcctggtcaaggactacttccccgaacccgtgaccgtgagctggaactcaggcgccctgaccagcggcgtgcacaccttccccgctgtcctgcagtcctcaggactctactccctcagcagcgtggtgaccgtgccctccagcagcttgggcacccagacctacatctgcaacgtgaatcacaagcccagcaacaccaaggtggacaagagagttgagcccaaatcttgtgacaaaactcacacatgcccaccctgcccagcacctgaagccgcggggggaccctcagtcttcctcttccccccaaaacccaaggacaccctcatgatctcccggacccctgaggtcacatgcgtggtggtggacgtgagccacgaagaccctgaggtcaagttcaactggtacgtggacggcgtggaggtgcataatgccaagacaaagccccgggaggagcagtacaacagcacgtaccgggtggtcagcgtcctcaccgtcctgcaccaggactggctgaatggcaaggagtacaagtgcaaggtctccaacaaagccctcccagcccccatcgagaaaaccatctccaaagccaaaggccagccccgggaaccacaggtgtacaccctgcccccatcccgggaggagatgaccaagaaccaggtcagcctgacctgcctggtcaaaggcttctatcccagcgacatcgccgtggagtgggagagcaatggccagcccgagaacaactacaagaccacccctcccgtgctggactccgacggctccttcttcctctacagcaagctcaccgtggacaagagcaggtggcagcagggcaacgtcttctcatgctccgtgatgcatgaggctctgcacaaccactacacccagaagagcctctccctgtctcccggcaaa

SEQ ID NO: 58 - protein, 122 aa, Artificial Sequence
  humanized antibody
  MISC_FEATURE: amino acid sequence of variable region of humanized antibody heavy chain hH2
EVQLVQSGAEVKKPGASVKVSCKTSGYTFTEYTMHWVRQAPGKSLEWMGGVNPNSGDTSYAQKFQGRVTITADTSTSTAYMELSSLRSEDTAVYYCARPGGYDVGYYAMDYWGQGTLVTVSS

SEQ ID NO: 59 - DNA, 366 bp, Artificial Sequence
  humanized antibody
  misc_feature: nucleotide sequence encoding variable region of humanized antibody heavy chain hH2
gaagtgcagctggtgcagtctggcgccgaagtgaagaaaccaggcgccagcgtgaaggtgtcctgcaagaccagcggctacacctttaccgagtacaccatgcactgggtgcgccaggcccctggcaagagcctggaatggatgggcggcgtgaaccccaacagcggcgatacaagctacgcccagaaattccagggcagagtgaccatcaccgccgacaccagcacctccaccgcctacatggaactgagcagcctgcggagcgaggacaccgccgtgtactactgtgctagacctggcggctacgacgtgggctactacgccatggattactggggccagggcaccctcgtgaccgtcagctca

SEQ ID NO: 60 - protein, 471 aa, Artificial Sequence
  humanized antibody
  MISC_FEATURE: amino acid sequence of humanized antibody heavy chain hH3
MKHLWFFLLLVAAPRWVLSEVQLVQSGAEVKKPGASVKVSCKTSGYTFTEYTMHWVRQAPGQGLEWMGGVNPNSGDTSYAQKFQGRVTLTVDKSTSTAYMELSSLRSEDTAVYYCARPGGYDVGYYAMDYWGQGTLVTVSSASTKGPSVFPLAPSSKSTSGGTAALGCLVKDYFPEPVTVSWNSGALTSGVHTFPAVLQSSGLYSLSSVVTVPSSSLGTQTYICNVNHKPSNTKVDKRVEPKSCDKTHTCPPCPAPEAAGGPSVFLFPPKPKDTLMISRTPEVTCVVVDVSHEDPEVKFNWYVDGVEVHNAKTKPREEQYNSTYRVVSVLTVLHQDWLNGKEYKCKVSNKALPAPIEKTISKAKGQPREPQVYTLPPSREEMTKNQVSLTCLVKGFYPSDIAVEWESNGQPENNYKTTPPVLDSDGSFFLYSKLTVDKSRWQQGNVFSCSVMHEALHNHYTQKSLSLSPGK

SEQ ID NO: 61 - DNA, 1413 bp, Artificial Sequence
  humanized antibody
  misc_feature: nucleotide sequence encoding humanized antibody heavy chain hH3
atgaaacacctgtggttcttcctcctgctggtggcagctcccagatgggtgctgagcgaagtgcagctggtgcagtctggcgccgaagtgaagaaaccaggcgccagcgtgaaggtgtcctgcaagaccagcggctacacctttaccgagtacaccatgcactgggtgcgccaggctccaggccagggactggaatggatgggcggcgtgaaccccaacagcggcgatacaagctacgcccagaaattccagggcagagtgaccctgaccgtggacaagagcaccagcaccgcctacatggaactgagcagcctgcggagcgaggacaccgccgtgtactactgtgctagacctggcggctacgacgtgggctactacgccatggattactggggccagggcaccctcgtgaccgtcagctcagcctccaccaagggcccaagcgtcttccccctggcaccctcctccaagagcacctctggcggcacagccgccctgggctgcctggtcaaggactacttccccgaacccgtgaccgtgagctggaactcaggcgccctgaccagcggcgtgcacaccttccccgctgtcctgcagtcctcaggactctactccctcagcagcgtggtgaccgtgccctccagcagcttgggcacccagacctacatctgcaacgtgaatcacaagcccagcaacaccaaggtggacaagagagttgagcccaaatcttgtgacaaaactcacacatgcccaccctgcccagcacctgaagccgcggggggaccctcagtcttcctcttccccccaaaacccaaggacaccctcatgatctcccggacccctgaggtcacatgcgtggtggtggacgtgagccacgaagaccctgaggtcaagttcaactggtacgtggacggcgtggaggtgcataatgccaagacaaagccccgggaggagcagtacaacagcacgtaccgggtggtcagcgtcctcaccgtcctgcaccaggactggctgaatggcaaggagtacaagtgcaaggtctccaacaaagccctcccagcccccatcgagaaaaccatctccaaagccaaaggccagccccgggaaccacaggtgtacaccctgcccccatcccgggaggagatgaccaagaaccaggtcagcctgacctgcctggtcaaaggcttctatcccagcgacatcgccgtggagtgggagagcaatggccagcccgagaacaactacaagaccacccctcccgtgctggactccgacggctccttcttcctctacagcaagctcaccgtggacaagagcaggtggcagcagggcaacgtcttctcatgctccgtgatgcatgaggctctgcacaaccactacacccagaagagcctctccctgtctcccggcaaa

SEQ ID NO: 62 - protein, 122 aa, Artificial Sequence
  humanized antibody
  MISC_FEATURE: amino acid sequence of variable region of humanized antibody heavy chain hH3
EVQLVQSGAEVKKPGASVKVSCKTSGYTFTEYTMHWVRQAPGQGLEWMGGVNPNSGDTSYAQKFQGRVTLTVDKSTSTAYMELSSLRSEDTAVYYCARPGGYDVGYYAMDYWGQGTLVTVSS

SEQ ID NO: 63 - DNA, 366 bp, Artificial Sequence
  humanized antibody
  misc_feature: nucleotide sequence encoding variable region of humanized antibody heavy chain hH3
gaagtgcagctggtgcagtctggcgccgaagtgaagaaaccaggcgccagcgtgaaggtgtcctgcaagaccagcggctacacctttaccgagtacaccatgcactgggtgcgccaggctccaggccagggactggaatggatgggcggcgtgaaccccaacagcggcgatacaagctacgcccagaaattccagggcagagtgaccctgaccgtggacaagagcaccagcaccgcctacatggaactgagcagcctgcggagcgaggacaccgccgtgtactactgtgctagacctggcggctacgacgtgggctactacgccatggattactggggccagggcaccctcgtgaccgtcagctca

SEQ ID NO: 64 - protein, 214 aa, Artificial Sequence
  humanized antibody
  MISC_FEATURE: amino acid sequence of Trastuzumab light chain
DIQMTQSPSSLSASVGDRVTITCRASQDVNTAVAWYQQKPGKAPKLLIYSASFLYSGVPSRFSGSRSGTDFTLTISSLQPEDFATYYCQQHYTTPPTFGQGTKVEIKRTVAAPSVFIFPPSDEQLKSGTASVVCLLNNFYPREAKVQWKVDNALQSGNSQESVTEQDSKDSTYSLSSTLTLSKADYEKHKVYACEVTHQGLSSPVTKSFNRGEC

SEQ ID NO: 65 - protein, 450 aa, Artificial Sequence
  humanized antibody
  MISC_FEATURE: amino acid sequence of Trastuzumab heavy chain
EVQLVESGGGLVQPGGSLRLSCAASGFNIKDTYIHWVRQAPGKGLEWVARIYPTNGYTRYADSVKGRFTISADTSKNTAYLQMNSLRAEDTAVYYCSRWGGDGFYAMDYWGQGTLVTVSSASTKGPSVFPLAPSSKSTSGGTAALGCLVKDYFPEPVTVSWNSGALTSGVHTFPAVLQSSGLYSLSSVVTVPSSSLGTQTYICNVNHKPSNTKVDKKVEPKSCDKTHTCPPCPAPELLGGPSVFLFPPKPKDTLMISRTPEVTCVVVDVSHEDPEVKFNWYVDGVEVHNAKTKPREEQYNSTYRVVSVLTVLHQDWLNGKEYKCKVSNKALPAPIEKTISKAKGQPREPQVYTLPPSREEMTKNQVSLTCLVKGFYPSDIAVEWESNGQPENNYKTTPPVLDSDGSFFLYSKLTVDKSRWQQGNVFSCSVMHEALHNHYTQKSLSLSPGK

SEQ ID NO: 66 - protein, 234 aa, Artificial Sequence
  humanized antibody
  MISC_FEATURE: amino acid sequence of anti-LPS antibody (h#1G5-H1L1) light chain
MVLQTQVFISLLLWISGAYGDIVMTQSPDSLAVSLGERATINCKASENVGNSVSWYQQKPGQPPKLLIYGASNRYTGVPDRFSGSGSGTDFTLTISSLQAEDVAVYYCGQSYSYPYTFGQGTKVEIKRTVAAPSVFIFPPSDEQLKSGTASVVCLLNNFYPREAKVQWKVDNALQSGNSQESVTEQDSKDSTYSLSSTLTLSKADYEKHKVYACEVTHQGLSSPVTKSFNRGEC

SEQ ID NO: 67 - protein, 474 aa, Artificial Sequence
  humanized antibody
  MISC_FEATURE: amino acid sequence of anti-LPS antibody (h#1G5-H1L1) heavy chain
MKHLWFFLLLVAAPRWVLSQVQLVQSGAEVKKPGASVKVSCKASGYTFTSYWINWVRQAPGQGLEWMGNIYPGSSSINYNEKFKSRVTITADTSTSTAYMELSSLRSEDTAVYYCARTIYNYGSSGYNYAMDYWGQGTLVTVSSASTKGPSVFPLAPSSKSTSGGTAALGCLVKDYFPEPVTVSWNSGALTSGVHTFPAVLQSSGLYSLSSVVTVPSSSLGTQTYICNVNHKPSNTKVDKRVEPKSCDKTHTCPPCPAPELLGGPSVFLFPPKPKDTLMISRTPEVTCVVVDVSHEDPEVKFNWYVDGVEVHNAKTKPREEQYNSTYRVVSVLTVLHQDWLNGKEYKCKVSNKALPAPIEKTISKAKGQPREPQVYTLPPSREEMTKNQVSLTCLVKGFYPSDIAVEWESNGQPENNYKTTPPVLDSDGSFFLYSKLTVDKSRWQQGNVFSCSVMHEALHNHYTQKSLSLSPGK

SEQ ID NO: 68 - protein, 234 aa, Artificial Sequence
  humanized antibody
  MISC_FEATURE: amino acid sequence of anti-TROP2 antibody (hRS7) light chain
MVLQTQVFISLLLWISGAYGDIQLTQSPSSLSASVGDRVSITCKASQDVSIAVAWYQQKPGKAPKLLIYSASYRYTGVPDRFSGSGSGTDFTLTISSLQPEDFAVYYCQQHYITPLTFGAGTKVEIKRTVAAPSVFIFPPSDEQLKSGTASVVCLLNNFYPREAKVQWKVDNALQSGNSQESVTEQDSKDSTYSLSSTLTLSKADYEKHKVYACEVTHQGLSSPVTKSFNRGEC

SEQ ID NO: 69 - protein, 470 aa, Artificial Sequence
  humanized antibody
  MISC_FEATURE: amino acid sequence of anti-TROP2 antibody (hRS7) heavy chain
MKHLWFFLLLVAAPRWVLSQVQLQQSGSELKKPGASVKVSCKASGYTFTNYGMNWVKQAPGQGLKWMGWINTYTGEPTYTDDFKGRFAFSLDTSVSTAYLQISSLKADDTAVYFCARGGFGSSYWYFDVWGQGSLVTVSSASTKGPSVFPLAPSSKSTSGGTAALGCLVKDYFPEPVTVSWNSGALTSGVHTFPAVLQSSGLYSLSSVVTVPSSSLGTQTYICNVNHKPSNTKVDKRVEPKSCDKTHTCPPCPAPELLGGPSVFLFPPKPKDTLMISRTPEVTCVVVDVSHEDPEVKFNWYVDGVEVHNAKTKPREEQYNSTYRVVSVLTVLHQDWLNGKEYKCKVSNKALPAPIEKTISKAKGQPREPQVYTLPPSREEMTKNQVSLTCLVKGFYPSDIAVEWESNGQPENNYKTTPPVLDSDGSFFLYSKLTVDKSRWQQGNVFSCSVMHEALHNHYTQKSLSLSPGK

SEQ ID NO: 70 - protein, 240 aa, Artificial Sequence
  humanized antibody
  MISC_FEATURE: amino acid sequence of anti-CD98 antibody (hM23-H1L1) light chain
MVLQTQVFISLLLWISGAYGDIVMTQSPDSLAVSLGERATINCKSSQSLLYSSNQKNYLAWYQQKPGQPPKLLIYWASTRESGVPDRFSGSGSGTDFTLTISSLQAEDVAVYYCQRYYGYPWTFGQGTKVEIKRTVAAPSVFIFPPSDEQLKSGTASVVCLLNNFYPREAKVQWKVDNALQSGNSQESVTEQDSKDSTYSLSSTLTLSKADYEKHKVYACEVTHQGLSSPVTKSFNRGEC

SEQ ID NO: 71 - protein, 465 aa, Artificial Sequence
  humanized antibody
  MISC_FEATURE: amino acid sequence of anti-CD98 antibody (hM23-H1L1) heavy chain
MKHLWFFLLLVAAPRWVLSQVQLVQSGAEVKKPGASVKVSCKASGYAFSNYLIEWVRQAPGQGLEWMGVINPGSGVTNYNEKFKGRVTITADTSTSTAYMELSSLRSEDTAVYYCARAEAWFAYWGQGTLVTVSSASTKGPSVFPLAPSSKSTSGGTAALGCLVKDYFPEPVTVSWNSGALTSGVHTFPAVLQSSGLYSLSSVVTVPSSSLGTQTYICNVNHKPSNTKVDKRVEPKSCDKTHTCPPCPAPELLGGPSVFLFPPKPKDTLMISRTPEVTCVVVDVSHEDPEVKFNWYVDGVEVHNAKTKPREEQYNSTYRVVSVLTVLHQDWLNGKEYKCKVSNKALPAPIEKTISKAKGQPREPQVYTLPPSREEMTKNQVSLTCLVKGFYPSDIAVEWESNGQPENNYKTTPPVLDSDGSFFLYSKLTVDKSRWQQGNVFSCSVMHEALHNHYTQKSLSLSPGK

SEQ ID NO: 72 - DNA, 702 bp, Artificial Sequence
  humanized antibody
  misc_feature: nucleotide sequence encoding Trastuzumab mutant light chain
atggtgctgcagacccaggtgttcatctccctgctgctgtggatctccggcgcgtacggcgacatccagatgacacagagccctagcagcctgtctgccagcgtgggagacagagtgaccatcacctgtagagccagccaggacgtgaacacagccgtggcttggtatcagcagaagcctggcaaggcccctaagctgctgatctacagcgccagctttctgtacagcggcgtgcccagcagattcagcggctctagaagcggcaccgacttcaccctgaccataagcagtctgcagcccgaggacttcgccacctactactgtcagcagcactacaccacacctccaacctttggccagggcaccaaggtggaaatcaagcgtacggtggccgccccctccgtgttcatcttccccccctccgacgagcagctgaagtccggcaccgcctccgtggtgtgcctgctgaataacttctaccccagagaggccaaggtgcagtggaaggtggacaacgccctgcagtccgggaactcccaggagagcgtgaccgagcaggacagcaaggacagcacctacagcctgagcagcaccctgaccctgagcaaagccgactacgagaagcacaaggtgtacgcctgcgaggtgacccaccagggcctgagctcccccgtcaccaagagcttcaacaggggggagtgt

SEQ ID NO: 73 - protein, 234 aa, Artificial Sequence
  humanized antibody
  MISC_FEATURE: amino acid sequence of Trastuzumab mutant light chain
MVLQTQVFISLLLWISGAYGDIQMTQSPSSLSASVGDRVTITCRASQDVNTAVAWYQQKPGKAPKLLIYSASFLYSGVPSRFSGSRSGTDFTLTISSLQPEDFATYYCQQHYTTPPTFGQGTKVEIKRTVAAPSVFIFPPSDEQLKSGTASVVCLLNNFYPREAKVQWKVDNALQSGNSQESVTEQDSKDSTYSLSSTLTLSKADYEKHKVYACEVTHQGLSSPVTKSFNRGEC

SEQ ID NO: 74 - DNA, 1407 bp, Artificial Sequence
  humanized antibody
  misc_feature: nucleotide sequence encoding Trastuzumab mutant heavy chain
atgaaacacctgtggttcttcctcctgctggtggcagctcccagatgggtgctgagcgaggtgcagctggttgaatctggcggaggactggttcagcctggcggatctctgagactgtcttgtgccgccagcggcttcaacatcaaggacacctacatccactgggtccgacaggcccctggcaaaggacttgaatgggtcgccagaatctaccccaccaacggctacaccagatacgccgactctgtgaagggcagattcaccatcagcgccgacaccagcaagaacaccgcctacctgcagatgaacagcctgagagccgaggacaccgccgtgtactactgttctagatggggaggcgacggcttctacgccatggattattggggccagggcaccctggttaccgttagctcagcctccaccaagggcccaagcgtcttccccctggcaccctcctccaagagcacctctggcggcacagccgccctgggctgcctggtcaaggactacttccccgaacccgtgaccgtgagctggaactcaggcgccctgaccagcggcgtgcacaccttccccgctgtcctgcagtcctcaggactctactccctcagcagcgtggtgaccgtgccctccagcagcttgggcacccagacctacatctgcaacgtgaatcacaagcccagcaacaccaaggtggacaagagagttgagcccaaatcttgtgacaaaactcacacatgcccaccctgcccagcacctgaagccgcggggggaccctcagtcttcctcttccccccaaaacccaaggacaccctcatgatctcccggacccctgaggtcacatgcgtggtggtggacgtgagccacgaagaccctgaggtcaagttcaactggtacgtggacggcgtggaggtgcataatgccaagacaaagccccgggaggagcagtacaacagcacgtaccgggtggtcagcgtcctcaccgtcctgcaccaggactggctgaatggcaaggagtacaagtgcaaggtctccaacaaagccctcccagcccccatcgagaaaaccatctccaaagccaaaggccagccccgggaaccacaggtgtacaccctgcccccatcccgggaggagatgaccaagaaccaggtcagcctgacctgcctggtcaaaggcttctatcccagcgacatcgccgtggagtgggagagcaatggccagcccgagaacaactacaagaccacccctcccgtgctggactccgacggctccttcttcctctacagcaagctcaccgtggacaagagcaggtggcagcagggcaacgtcttctcatgctccgtgatgcatgaggctctgcacaaccactacacccagaagagcctctccctgtctcccggcaaa

SEQ ID NO: 75 - protein, 469 aa, Artificial Sequence
  humanized antibody
  MISC_FEATURE: amino acid sequence of Trastuzumab mutant heavy chain
MKHLWFFLLLVAAPRWVLSEVQLVESGGGLVQPGGSLRLSCAASGFNIKDTYIHWVRQAPGKGLEWVARIYPTNGYTRYADSVKGRFTISADTSKNTAYLQMNSLRAEDTAVYYCSRWGGDGFYAMDYWGQGTLVTVSSASTKGPSVFPLAPSSKSTSGGTAALGCLVKDYFPEPVTVSWNSGALTSGVHTFPAVLQSSGLYSLSSVVTVPSSSLGTQTYICNVNHKPSNTKVDKRVEPKSCDKTHTCPPCPAPEAAGGPSVFLFPPKPKDTLMISRTPEVTCVVVDVSHEDPEVKFNWYVDGVEVHNAKTKPREEQYNSTYRVVSVLTVLHQDWLNGKEYKCKVSNKALPAPIEKTISKAKGQPREPQVYTLPPSREEMTKNQVSLTCLVKGFYPSDIAVEWESNGQPENNYKTTPPVLDSDGSFFLYSKLTVDKSRWQQGNVFSCSVMHEALHNHYTQKSLSLSPGK